European Patent Application EP 4 273 240 A1, published November 8, 2023. Title: method for gene function regulation by a novel guide nucleic acid mechanism. Applicant: Kobe University. The sequence listing filed with the application follows.

SEQUENCE LISTING (28 sequences)

SEQ ID NO: 1 - DNA, 7934 bp, Artificial Sequence
  pT7SU_RsAgo
agatctcgatcccgcgaaattaatacgactcactataggggaattgtgagcggataacaattcccctctagaaataattttgtttaactttaagaaggagatataccatgggtcatcaccatcatcatcacgggtccctgcaggactcagaagtcaatcaagaagctaagccagaggtcaagccagaagtcaagcctgagactcacatcaatttaaaggtgtccgatggatcttcagagatcttcttcaagatcaaaaagaccactcctttaagaaggctgatggaagcgttcgctaaaagacagggtaaggaaatggactccttaagattcttgtacgacggtattagaattcaagctgatcaggcccctgaagatttggacatggaggataacgatattattgaggctcaccgcgaacagattggaggtgcaccagtccaggcagcagatgagatgtatgatagcaacccacacccagacagacgccagctggtgagcaacggcttcgaagtgaatctgcccgatcaggtggaggtcatcgtgcgggacctgccagatcccagtaaggtgaaagaggaacgaacccggctgatggggtactggttcgtgcactggtttgatggaaagctgtttcatctgagaatcaaagcaggaggaccaaacgtggacggagaacacagggccattcgcacagctgagcatccctggctgctgagagctaggctggacgatgcactggaggaagccctgcctaagtatgccgctgtgaagaaaaggccattcacatttctggcccagaaagacgaactgatcgatgcagccgctactgcagccggactgagccacagactgctgaatagcttcaaagtgatccctaggtttgccctgagcccaaaaatctacgagccagtggacggaaccacacgcgtcggcgtgttcgtcaccatcggcatgcggtatgacattgaagccagcctgagagatctgctggaggctgggatcgacctgcggggaatgtacgtggtccggagaaagcgacagccaggggagcgaggactgctgggacgcgtccgagccattagcgacgatatggtgcagctgttcgaggaaaccgatctggcttccgtgaacgtcaatgacgcaaagctggaaggctccaaagagaactttacaagatgcctgtctgccctgctggggcataactacaagaaactgctgaatgctctggacgatcaggaagcagggtatcgcacaggacctcgattcgacgatgcagtgaggcgcatgggcgagtttctggccaagaaaccaatcagactggctgataacattaatgcacaagtgggcgacaggatcgtcttcagcaacgagggacaggcacgaaatgtgcggctggctcccaaggtggaatacgtctttgataggactggggcaaaaagtgccgagtatgcttggcgcggcctgtcacagttcgggccttttgaccggccatccttcgccaacagatctccaaggattctggtggtctaccccagctccacacagggcaaggtggagaacttcctgagcgcctttagagatggaatgggcagtaattattcaggcttcagcaaggggtttgtggacctgatggggctgacaaaagtggaattcgtcatgtgccctgtggaggtgagcagcgccgataggaacggcgcccacactaagtacaattccgccatcgaagacaaactggcaggagctggagaggtgcacgctggaattgtggtcctgtttgaggaccatgcaagactgcctgacgataggaatccatatatccatacaaagtctctgctgctgacactgggggtgccaactcagcaggtccgcatgcccactgtgctgctggaacctaaaagcctgcagtacactctgcagaacttctccatcgcaacctatgccaagctgaatggcacaccctggactgtgaaccacgacaaagctattaatgatgagctggtggtcggcatggggctggcagaactgtcagggagccggaccgagaagcggcagagattcgtcggaatcactaccgtgtttgccggagatggctcatacctgctgggaaacgtgagcaaagagtgcgaatacgagggctattctgacgctatcagggaaagtatgactggaattctgcgcgagctgaagaaacggaacaattggcggcccggcgacaccgtgagagtggtcttccacgcccataggcctctgaagcgcgtggatgtcgcttcaatcgtgtttgaatgtaccagggagatcggcagcgaccagaatattcagatggccttcgtgacagtctcccacgatcatccctttgtgctgattgaccgctctgaacgaggactggaggcatataagggcagtactgcccgaaaaggggtgttcgcaccacctcggggagcaatcagtcgggtcggcagactgaccaggctgctggcagtgaactcaccccagctgattaagcgcgccaatactcctctgccaacccccctgctggtcagtctgcaccctgactcaaccttcaaggacgtggattacctggctgagcaggccctgaagttcacctccctgtcttggcggtctacactgcccgctgcaacccctgtgacaatcttttattccgaacgcattgccgagctgctgggccgactgaagtctattcctaactggtcatccgccaatctgaacatcaagctgaagtggagcaggtggtttctgtgatctagaggatccgaattcgagctccgtcgacaagcttgcggccgcactcgagcaccaccaccaccaccactgagatccggctgctaacaaagcccgaaaggaagctgagttggctgctgccaccgctgagcaataactagcataaccccttggggcctctaaacgggtcttgaggggttttttgctgaaaggaggaactatatccggattggcgaatgggacgcgccctgtagcggcgcattaagcgcggcgggtgtggtggttacgcgcagcgtgaccgctacacttgccagcgccctagcgcccgctcctttcgctttcttcccttcctttctcgccacgttcgccggctttccccgtcaagctctaaatcgggggctccctttagggttccgatttagtgctttacggcacctcgaccccaaaaaacttgattagggtgatggttcacgtagtgggccatcgccctgatagacggtttttcgccctttgacgttggagtccacgttctttaatagtggactcttgttccaaactggaacaacactcaaccctatctcggtctattcttttgatttataagggattttgccgatttcggcctattggttaaaaaatgagctgatttaacaaaaatttaacgcgaattttaacaaaatattaacgtttacaatttcaggtggcacttttcggggaaatgtgcgcggaacccctatttgtttatttttctaaatacattcaaatatgtatccgctcatgaattaattcttagaaaaactcatcgagcatcaaatgaaactgcaatttattcatatcaggattatcaataccatatttttgaaaaagccgtttctgtaatgaaggagaaaactcaccgaggcagttccataggatggcaagatcctggtatcggtctgcgattccgactcgtccaacatcaatacaacctattaatttcccctcgtcaaaaataaggttatcaagtgagaaatcaccatgagtgacgactgaatccggtgagaatggcaaaagtttatgcatttctttccagacttgttcaacaggccagccattacgctcgtcatcaaaatcactcgcatcaaccaaaccgttattcattcgtgattgcgcctgagcgagacgaaatacgcgatcgctgttaaaaggacaattacaaacaggaatcgaatgcaaccggcgcaggaacactgccagcgcatcaacaatattttcacctgaatcaggatattcttctaatacctggaatgctgttttcccggggatcgcagtggtgagtaaccatgcatcatcaggagtacggataaaatgcttgatggtcggaagaggcataaattccgtcagccagtttagtctgaccatctcatctgtaacatcattggcaacgctacctttgccatgtttcagaaacaactctggcgcatcgggcttcccatacaatcgatagattgtcgcacctgattgcccgacattatcgcgagcccatttatacccatataaatcagcatccatgttggaatttaatcgcggcctagagcaagacgtttcccgttgaatatggctcataacaccccttgtattactgtttatgtaagcagacagttttattgttcatgaccaaaatcccttaacgtgagttttcgttccactgagcgtcagaccccgtagaaaagatcaaaggatcttcttgagatcctttttttctgcgcgtaatctgctgcttgcaaacaaaaaaaccaccgctaccagcggtggtttgtttgccggatcaagagctaccaactctttttccgaaggtaactggcttcagcagagcgcagataccaaatactgtccttctagtgtagccgtagttaggccaccacttcaagaactctgtagcaccgcctacatacctcgctctgctaatcctgttaccagtggctgctgccagtggcgataagtcgtgtcttaccgggttggactcaagacgatagttaccggataaggcgcagcggtcgggctgaacggggggttcgtgcacacagcccagcttggagcgaacgacctacaccgaactgagatacctacagcgtgagctatgagaaagcgccacgcttcccgaagggagaaaggcggacaggtatccggtaagcggcagggtcggaacaggagagcgcacgagggagcttccagggggaaacgcctggtatctttatagtcctgtcgggtttcgccacctctgacttgagcgtcgatttttgtgatgctcgtcaggggggcggagcctatggaaaaacgccagcaacgcggcctttttacggttcctggccttttgctggccttttgctcacatgttctttcctgcgttatcccctgattctgtggataaccgtattaccgcctttgagtgagctgataccgctcgccgcagccgaacgaccgagcgcagcgagtcagtgagcgaggaagcggaagagcgcctgatgcggtattttctccttacgcatctgtgcggtatttcacaccgcatatatggtgcactctcagtacaatctgctctgatgccgcatagttaagccagtatacactccgctatcgctacgtgactgggtcatggctgcgccccgacacccgccaacacccgctgacgcgccctgacgggcttgtctgctcccggcatccgcttacagacaagctgtgaccgtctccgggagctgcatgtgtcagaggttttcaccgtcatcaccgaaacgcgcgaggcagctgcggtaaagctcatcagcgtggtcgtgaagcgattcacagatgtctgcctgttcatccgcgtccagctcgttgagtttctccagaagcgttaatgtctggcttctgataaagcgggccatgttaagggcggttttttcctgtttggtcactgatgcctccgtgtaagggggatttctgttcatgggggtaatgataccgatgaaacgagagaggatgctcacgatacgggttactgatgatgaacatgcccggttactggaacgttgtgagggtaaacaactggcggtatggatgcggcgggaccagagaaaaatcactcagggtcaatgccagcgcttcgttaatacagatgtaggtgttccacagggtagccagcagcatcctgcgatgcagatccggaacataatggtgcagggcgctgacttccgcgtttccagactttacgaaacacggaaaccgaagaccattcatgttgttgctcaggtcgcagacgttttgcagcagcagtcgcttcacgttcgctcgcgtatcggtgattcattctgctaaccagtaaggcaaccccgccagcctagccgggtcctcaacgacaggagcacgatcatgcgcacccgtggggccgccatgccggcgataatggcctgcttctcgccgaaacgtttggtggcgggaccagtgacgaaggcttgagcgagggcgtgcaagattccgaataccgcaagcgacaggccgatcatcgtcgcgctccagcgaaagcggtcctcgccgaaaatgacccagagcgctgccggcacctgtcctacgagttgcatgataaagaagacagtcataagtgcggcgacgatagtcatgccccgcgcccaccggaaggagctgactgggttgaaggctctcaagggcatcggtcgagatcccggtgcctaatgagtgagctaacttacattaattgcgttgcgctcactgcccgctttccagtcgggaaacctgtcgtgccagctgcattaatgaatcggccaacgcgcggggagaggcggtttgcgtattgggcgccagggtggtttttcttttcaccagtgagacgggcaacagctgattgcccttcaccgcctggccctgagagagttgcagcaagcggtccacgctggtttgccccagcaggcgaaaatcctgtttgatggtggttaacggcgggatataacatgagctgtcttcggtatcgtcgtatcccactaccgagatatccgcaccaacgcgcagcccggactcggtaatggcgcgcattgcgcccagcgccatctgatcgttggcaaccagcatcgcagtgggaacgatgccctcattcagcatttgcatggtttgttgaaaaccggacatggcactccagtcgccttcccgttccgctatcggctgaatttgattgcgagtgagatatttatgccagccagccagacgcagacgcgccgagacagaacttaatgggcccgctaacagcgcgatttgctggtgacccaatgcgaccagatgctccacgcccagtcgcgtaccgtcttcatgggagaaaataatactgttgatgggtgtctggtcagagacatcaagaaataacgccggaacattagtgcaggcagcttccacagcaatggcatcctggtcatccagcggatagttaatgatcagcccactgacgcgttgcgcgagaagattgtgcaccgccgctttacaggcttcgacgccgcttcgttctaccatcgacaccaccacgctggcacccagttgatcggcgcgagatttaatcgccgcgacaatttgcgacggcgcgtgcagggccagactggaggtggcaacgccaatcagcaacgactgtttgcccgccagttgttgtgccacgcggttgggaatgtaattcagctccgccatcgccgcttccactttttcccgcgttttcgcagaaacgtggctggcctggttcaccacgcgggaaacggtctgataagagacaccggcatactctgcgacatcgtataacgttactggtttcacattcaccaccctgaattgactctcttccgggcgctatcatgccataccgcgaaaggttttgcgccattcgatggtgtccgggatctcgacgctctcccttatgcgactcctgcattaggaagcagcccagtagtaggttgaggccgttgagcaccgccgccgcaaggaatggtgcatgcaaggagatggcgcccaacagtcccccggccacggggcctgccaccatacccacgccgaaacaagcgctcatgagcccgaagtggcgagcccgatcttccccatcggtgatgtcggcgatataggcgccagcaaccgcacctgtggcgccggtgatgccggccacgatgcgtccggcgtagaggatcg

SEQ ID NO: 2 - RNA, 18 nt, Artificial Sequence
  Synthetic RNA used in Example 2
uuacaaccuacuaccucg

SEQ ID NO: 3 - DNA, 18 bp, Artificial Sequence
  Synthetic DNA used in Example 2.
cgaggtagtaggttgtaa

SEQ ID NO: 4 - RNA, 18 nt, Artificial Sequence
  Synthetic RNA used in Example 3
uuacaaccuacuaccucg

SEQ ID NO: 5 - DNA, 20 bp, Artificial Sequence
  Synthetic DNA used in Example 3
cgaggtagtaggttgtaact

SEQ ID NO: 6 - DNA, 30 bp, Artificial Sequence
  Synthetic DNA used in Example 3
cccatgcgaggtagtaggttgtaactagag

SEQ ID NO: 7 - DNA, 40 bp, Artificial Sequence
  Synthetic DNA used in Example 3
gatgacccatgcgaggtagtaggttgtaactagaggggaa

SEQ ID NO: 8 - DNA, 42 bp, Artificial Sequence
  Synthetic DNA used in Example 3
taagaaggagatataccatggacaagaagtactccattgggc

SEQ ID NO: 9 - DNA, 22 bp, Artificial Sequence
  Synthetic DNA described  in Fig 7
taatacgactcactatagggtt

SEQ ID NO: 10 - DNA, 22 bp, Artificial Sequence
  Synthetic DNA described in Fig 7
attatgctgagtgatatcccaa

SEQ ID NO: 11 - DNA, 20 bp, Artificial Sequence
  Synthetic DNA used in Fig 7
taatacgactcactataggg

SEQ ID NO: 12 - DNA, 20 bp, Artificial Sequence
  Synthetic DNA used in Fig 7
attatgctgagtgatatccc

SEQ ID NO: 13 - RNA, 48 nt, Artificial Sequence
  guide RNA described in Fig 8
uuguaacuaugaguccgugaggacgaaacgaguaagcucgucuuacaa

SEQ ID NO: 14 - RNA, 42 nt, Artificial Sequence
  guide RNA described  in Fig 8
uuguaacuaugaguccgugaggacgaaacgaguaagcucguc

SEQ ID NO: 15 - RNA, 18 nt, Artificial Sequence
  Synthetic RNA used in Example 6
uuacaaccuacuaccucg

SEQ ID NO: 16 - DNA, 5198 bp, Artificial Sequence
  pHMk047_pT7_HH-hm014-MS2 template
agatctcgatcccgcgaaattaatacgactcactatagggggttgtaactgatgagtccgtgaggacgaaacgagtaagctcgtcttacaacctactacctcggggagcacatgaggatcacccatgtgcgactcccacagtcactggggagtcttcccgggctagcataaccccttggggcctctaaacgggtcttgaggggttttttgctgaaaggaggaactatatccggattggcgaatgggacgcgccctgtagcggcgcattaagcgcggcgggtgtggtggttacgcgcagcgtgaccgctacacttgccagcgccctagcgcccgctcctttcgctttcttcccttcctttctcgccacgttcgccggctttccccgtcaagctctaaatcgggggctccctttagggttccgatttagtgctttacggcacctcgaccccaaaaaacttgattagggtgatggttcacgtagtgggccatcgccctgatagacggtttttcgccctttgacgttggagtccacgttctttaatagtggactcttgttccaaactggaacaacactcaaccctatctcggtctattcttttgatttataagggattttgccgatttcggcctattggttaaaaaatgagctgatttaacaaaaatttaacgcgaattttaacaaaatattaacgtttacaatttcaggtggcacttttcggggaaatgtgcgcggaacccctatttgtttatttttctaaatacattcaaatatgtatccgctcatgaattaattcttagaaaaactcatcgagcatcaaatgaaactgcaatttattcatatcaggattatcaataccatatttttgaaaaagccgtttctgtaatgaaggagaaaactcaccgaggcagttccataggatggcaagatcctggtatcggtctgcgattccgactcgtccaacatcaatacaacctattaatttcccctcgtcaaaaataaggttatcaagtgagaaatcaccatgagtgacgactgaatccggtgagaatggcaaaagtttatgcatttctttccagacttgttcaacaggccagccattacgctcgtcatcaaaatcactcgcatcaaccaaaccgttattcattcgtgattgcgcctgagcgagacgaaatacgcgatcgctgttaaaaggacaattacaaacaggaatcgaatgcaaccggcgcaggaacactgccagcgcatcaacaatattttcacctgaatcaggatattcttctaatacctggaatgctgttttcccggggatcgcagtggtgagtaaccatgcatcatcaggagtacggataaaatgcttgatggtcggaagaggcataaattccgtcagccagtttagtctgaccatctcatctgtaacatcattggcaacgctacctttgccatgtttcagaaacaactctggcgcatcgggcttcccatacaatcgatagattgtcgcacctgattgcccgacattatcgcgagcccatttatacccatataaatcagcatccatgttggaatttaatcgcggcctagagcaagacgtttcccgttgaatatggctcataacaccccttgtattactgtttatgtaagcagacagttttattgttcatgaccaaaatcccttaacgtgagttttcgttccactgagcgtcagaccccgtagaaaagatcaaaggatcttcttgagatcctttttttctgcgcgtaatctgctgcttgcaaacaaaaaaaccaccgctaccagcggtggtttgtttgccggatcaagagctaccaactctttttccgaaggtaactggcttcagcagagcgcagataccaaatactgtccttctagtgtagccgtagttaggccaccacttcaagaactctgtagcaccgcctacatacctcgctctgctaatcctgttaccagtggctgctgccagtggcgataagtcgtgtcttaccgggttggactcaagacgatagttaccggataaggcgcagcggtcgggctgaacggggggttcgtgcacacagcccagcttggagcgaacgacctacaccgaactgagatacctacagcgtgagctatgagaaagcgccacgcttcccgaagggagaaaggcggacaggtatccggtaagcggcagggtcggaacaggagagcgcacgagggagcttccagggggaaacgcctggtatctttatagtcctgtcgggtttcgccacctctgacttgagcgtcgatttttgtgatgctcgtcaggggggcggagcctatggaaaaacgccagcaacgcggcctttttacggttcctggccttttgctggccttttgctcacatgttctttcctgcgttatcccctgattctgtggataaccgtattaccgcctttgagtgagctgataccgctcgccgcagccgaacgaccgagcgcagcgagtcagtgagcgaggaagcggaagagcgcctgatgcggtattttctccttacgcatctgtgcggtatttcacaccgcatatatggtgcactctcagtacaatctgctctgatgccgcatagttaagccagtatacactccgctatcgctacgtgactgggtcatggctgcgccccgacacccgccaacacccgctgacgcgccctgacgggcttgtctgctcccggcatccgcttacagacaagctgtgaccgtctccgggagctgcatgtgtcagaggttttcaccgtcatcaccgaaacgcgcgaggcagctgcggtaaagctcatcagcgtggtcgtgaagcgattcacagatgtctgcctgttcatccgcgtccagctcgttgagtttctccagaagcgttaatgtctggcttctgataaagcgggccatgttaagggcggttttttcctgtttggtcactgatgcctccgtgtaagggggatttctgttcatgggggtaatgataccgatgaaacgagagaggatgctcacgatacgggttactgatgatgaacatgcccggttactggaacgttgtgagggtaaacaactggcggtatggatgcggcgggaccagagaaaaatcactcagggtcaatgccagcgcttcgttaatacagatgtaggtgttccacagggtagccagcagcatcctgcgatgcagatccggaacataatggtgcagggcgctgacttccgcgtttccagactttacgaaacacggaaaccgaagaccattcatgttgttgctcaggtcgcagacgttttgcagcagcagtcgcttcacgttcgctcgcgtatcggtgattcattctgctaaccagtaaggcaaccccgccagcctagccgggtcctcaacgacaggagcacgatcatgcgcacccgtggggccgccatgccggcgataatggcctgcttctcgccgaaacgtttggtggcgggaccagtgacgaaggcttgagcgagggcgtgcaagattccgaataccgcaagcgacaggccgatcatcgtcgcgctccagcgaaagcggtcctcgccgaaaatgacccagagcgctgccggcacctgtcctacgagttgcatgataaagaagacagtcataagtgcggcgacgatagtcatgccccgcgcccaccggaaggagctgactgggttgaaggctctcaagggcatcggtcgagatcccggtgcctaatgagtgagctaacttacattaattgcgttgcgctcactgcccgctttccagtcgggaaacctgtcgtgccagctgcattaatgaatcggccaacgcgcggggagaggcggtttgcgtattgggcgccagggtggtttttcttttcaccagtgagacgggcaacagctgattgcccttcaccgcctggccctgagagagttgcagcaagcggtccacgctggtttgccccagcaggcgaaaatcctgtttgatggtggttaacggcgggatataacatgagctgtcttcggtatcgtcgtatcccactaccgagatatccgcaccaacgcgcagcccggactcggtaatggcgcgcattgcgcccagcgccatctgatcgttggcaaccagcatcgcagtgggaacgatgccctcattcagcatttgcatggtttgttgaaaaccggacatggcactccagtcgccttcccgttccgctatcggctgaatttgattgcgagtgagatatttatgccagccagccagacgcagacgcgccgagacagaacttaatgggcccgctaacagcgcgatttgctggtgacccaatgcgaccagatgctccacgcccagtcgcgtaccgtcttcatgggagaaaataatactgttgatgggtgtctggtcagagacatcaagaaataacgccggaacattagtgcaggcagcttccacagcaatggcatcctggtcatccagcggatagttaatgatcagcccactgacgcgttgcgcgagaagattgtgcaccgccgctttacaggcttcgacgccgcttcgttctaccatcgacaccaccacgctggcacccagttgatcggcgcgagatttaatcgccgcgacaatttgcgacggcgcgtgcagggccagactggaggtggcaacgccaatcagcaacgactgtttgcccgccagttgttgtgccacgcggttgggaatgtaattcagctccgccatcgccgcttccactttttcccgcgttttcgcagaaacgtggctggcctggttcaccacgcgggaaacggtctgataagagacaccggcatactctgcgacatcgtataacgttactggtttcacattcaccaccctgaattgactctcttccgggcgctatcatgccataccgcgaaaggttttgcgccattcgatggtgtccgggatctcgacgctctcccttatgcgactcctgcattaggaagcagcccagtagtaggttgaggccgttgagcaccgccgccgcaaggaatggtgcatgcaaggagatggcgcccaacagtcccccggccacggggcctgccaccatacccacgccgaaacaagcgctcatgagcccgaagtggcgagcccgatcttccccatcggtgatgtcggcgatataggcgccagcaaccgcacctgtggcgccggtgatgccggccacgatgcgtccggcgtagaggatcg

SEQ ID NO: 17 - DNA, 58 bp, Artificial Sequence
  Synthetic DNA used in Example 6
ggataacaattcccctctagaagtggttcgtgcttcaacatgggtcatcaccatcatc

SEQ ID NO: 18 - DNA, 58 bp, Artificial Sequence
  Synthetic DNA used in Example 6
gatgatggtgatgacccatgcgaggtagtaggttgtaactagaggggaattgttatcc

SEQ ID NO: 19 - DNA, 58 bp, Artificial Sequence
  Synthetic DNA used in Example 6
ggataacaattcccctctagttacaacctactacctcgcatgggtcatcaccatcatc

SEQ ID NO: 20 - DNA, 58 bp, Artificial Sequence; identical to SEQ ID NO: 18
  Synthetic DNA used in Example 6

SEQ ID NO: 21 - DNA, 58 bp, Artificial Sequence
  Synthetic DNA used in Example 7
ggataacaattcccctctagaagtggttcgctacctcgcatgggtcatcaccatcatc

SEQ ID NO: 22 - DNA, 58 bp, Artificial Sequence; identical to SEQ ID NO: 18
  Synthetic DNA used in Example 7

SEQ ID NO: 23 - DNA, 58 bp, Artificial Sequence
  Synthetic DNA used in Example 7
ggataacaattcccctctagttacaacccgtgcttcaacatgggtcatcaccatcatc

SEQ ID NO: 24 - DNA, 58 bp, Artificial Sequence; identical to SEQ ID NO: 18
  Synthetic DNA used in Example 7

SEQ ID NO: 25 - DNA, 73 bp, Artificial Sequence
  guide RNA aptamar used in Example 8
ttacaacctactacctcggggagcacatgaggatcacccatgtgcgactcccacagtcactggggagtcttcc

SEQ ID NO: 26 - DNA, 73 bp, Artificial Sequence
  guide RNA aptamar used in Example 8
cgaggtagtaggttgtaagggagcacatgaggatcacccatgtgcgactcccacagtcactggggagtcttcc

SEQ ID NO: 27 - DNA, 5611 bp, Artificial Sequence
  pHMk016_pT7SU+hm014 target
agatctcgatcccgcgaaattaatacgactcactataggggaattgtgagcggataacaattcccctctagttacaacctactacctcgcatgggtcatcaccatcatcatcacgggtccctgcaggactcagaagtcaatcaagaagctaagccagaggtcaagccagaagtcaagcctgagactcacatcaatttaaaggtgtccgatggatcttcagagatcttcttcaagatcaaaaagaccactcctttaagaaggctgatggaagcgttcgctaaaagacagggtaaggaaatggactccttaagattcttgtacgacggtattagaattcaagctgatcaggcccctgaagatttggacatggaggataacgatattattgaggctcaccgcgaacagattggaggttgagaccactagtggtaccggtctcactagaggatccgaattcgagctccgtcgacaagcttgcggccgcactcgagcaccaccaccaccaccactgagatccggctgctaacaaagcccgaaaggaagctgagttggctgctgccaccgctgagcaataactagcataaccccttggggcctctaaacgggtcttgaggggttttttgctgaaaggaggaactatatccggattggcgaatgggacgcgccctgtagcggcgcattaagcgcggcgggtgtggtggttacgcgcagcgtgaccgctacacttgccagcgccctagcgcccgctcctttcgctttcttcccttcctttctcgccacgttcgccggctttccccgtcaagctctaaatcgggggctccctttagggttccgatttagtgctttacggcacctcgaccccaaaaaacttgattagggtgatggttcacgtagtgggccatcgccctgatagacggtttttcgccctttgacgttggagtccacgttctttaatagtggactcttgttccaaactggaacaacactcaaccctatctcggtctattcttttgatttataagggattttgccgatttcggcctattggttaaaaaatgagctgatttaacaaaaatttaacgcgaattttaacaaaatattaacgtttacaatttcaggtggcacttttcggggaaatgtgcgcggaacccctatttgtttatttttctaaatacattcaaatatgtatccgctcatgaattaattcttagaaaaactcatcgagcatcaaatgaaactgcaatttattcatatcaggattatcaataccatatttttgaaaaagccgtttctgtaatgaaggagaaaactcaccgaggcagttccataggatggcaagatcctggtatcggtctgcgattccgactcgtccaacatcaatacaacctattaatttcccctcgtcaaaaataaggttatcaagtgagaaatcaccatgagtgacgactgaatccggtgagaatggcaaaagtttatgcatttctttccagacttgttcaacaggccagccattacgctcgtcatcaaaatcactcgcatcaaccaaaccgttattcattcgtgattgcgcctgagcgagacgaaatacgcgatcgctgttaaaaggacaattacaaacaggaatcgaatgcaaccggcgcaggaacactgccagcgcatcaacaatattttcacctgaatcaggatattcttctaatacctggaatgctgttttcccggggatcgcagtggtgagtaaccatgcatcatcaggagtacggataaaatgcttgatggtcggaagaggcataaattccgtcagccagtttagtctgaccatctcatctgtaacatcattggcaacgctacctttgccatgtttcagaaacaactctggcgcatcgggcttcccatacaatcgatagattgtcgcacctgattgcccgacattatcgcgagcccatttatacccatataaatcagcatccatgttggaatttaatcgcggcctagagcaagacgtttcccgttgaatatggctcataacaccccttgtattactgtttatgtaagcagacagttttattgttcatgaccaaaatcccttaacgtgagttttcgttccactgagcgtcagaccccgtagaaaagatcaaaggatcttcttgagatcctttttttctgcgcgtaatctgctgcttgcaaacaaaaaaaccaccgctaccagcggtggtttgtttgccggatcaagagctaccaactctttttccgaaggtaactggcttcagcagagcgcagataccaaatactgtccttctagtgtagccgtagttaggccaccacttcaagaactctgtagcaccgcctacatacctcgctctgctaatcctgttaccagtggctgctgccagtggcgataagtcgtgtcttaccgggttggactcaagacgatagttaccggataaggcgcagcggtcgggctgaacggggggttcgtgcacacagcccagcttggagcgaacgacctacaccgaactgagatacctacagcgtgagctatgagaaagcgccacgcttcccgaagggagaaaggcggacaggtatccggtaagcggcagggtcggaacaggagagcgcacgagggagcttccagggggaaacgcctggtatctttatagtcctgtcgggtttcgccacctctgacttgagcgtcgatttttgtgatgctcgtcaggggggcggagcctatggaaaaacgccagcaacgcggcctttttacggttcctggccttttgctggccttttgctcacatgttctttcctgcgttatcccctgattctgtggataaccgtattaccgcctttgagtgagctgataccgctcgccgcagccgaacgaccgagcgcagcgagtcagtgagcgaggaagcggaagagcgcctgatgcggtattttctccttacgcatctgtgcggtatttcacaccgcatatatggtgcactctcagtacaatctgctctgatgccgcatagttaagccagtatacactccgctatcgctacgtgactgggtcatggctgcgccccgacacccgccaacacccgctgacgcgccctgacgggcttgtctgctcccggcatccgcttacagacaagctgtgaccgtctccgggagctgcatgtgtcagaggttttcaccgtcatcaccgaaacgcgcgaggcagctgcggtaaagctcatcagcgtggtcgtgaagcgattcacagatgtctgcctgttcatccgcgtccagctcgttgagtttctccagaagcgttaatgtctggcttctgataaagcgggccatgttaagggcggttttttcctgtttggtcactgatgcctccgtgtaagggggatttctgttcatgggggtaatgataccgatgaaacgagagaggatgctcacgatacgggttactgatgatgaacatgcccggttactggaacgttgtgagggtaaacaactggcggtatggatgcggcgggaccagagaaaaatcactcagggtcaatgccagcgcttcgttaatacagatgtaggtgttccacagggtagccagcagcatcctgcgatgcagatccggaacataatggtgcagggcgctgacttccgcgtttccagactttacgaaacacggaaaccgaagaccattcatgttgttgctcaggtcgcagacgttttgcagcagcagtcgcttcacgttcgctcgcgtatcggtgattcattctgctaaccagtaaggcaaccccgccagcctagccgggtcctcaacgacaggagcacgatcatgcgcacccgtggggccgccatgccggcgataatggcctgcttctcgccgaaacgtttggtggcgggaccagtgacgaaggcttgagcgagggcgtgcaagattccgaataccgcaagcgacaggccgatcatcgtcgcgctccagcgaaagcggtcctcgccgaaaatgacccagagcgctgccggcacctgtcctacgagttgcatgataaagaagacagtcataagtgcggcgacgatagtcatgccccgcgcccaccggaaggagctgactgggttgaaggctctcaagggcatcggtcgagatcccggtgcctaatgagtgagctaacttacattaattgcgttgcgctcactgcccgctttccagtcgggaaacctgtcgtgccagctgcattaatgaatcggccaacgcgcggggagaggcggtttgcgtattgggcgccagggtggtttttcttttcaccagtgagacgggcaacagctgattgcccttcaccgcctggccctgagagagttgcagcaagcggtccacgctggtttgccccagcaggcgaaaatcctgtttgatggtggttaacggcgggatataacatgagctgtcttcggtatcgtcgtatcccactaccgagatatccgcaccaacgcgcagcccggactcggtaatggcgcgcattgcgcccagcgccatctgatcgttggcaaccagcatcgcagtgggaacgatgccctcattcagcatttgcatggtttgttgaaaaccggacatggcactccagtcgccttcccgttccgctatcggctgaatttgattgcgagtgagatatttatgccagccagccagacgcagacgcgccgagacagaacttaatgggcccgctaacagcgcgatttgctggtgacccaatgcgaccagatgctccacgcccagtcgcgtaccgtcttcatgggagaaaataatactgttgatgggtgtctggtcagagacatcaagaaataacgccggaacattagtgcaggcagcttccacagcaatggcatcctggtcatccagcggatagttaatgatcagcccactgacgcgttgcgcgagaagattgtgcaccgccgctttacaggcttcgacgccgcttcgttctaccatcgacaccaccacgctggcacccagttgatcggcgcgagatttaatcgccgcgacaatttgcgacggcgcgtgcagggccagactggaggtggcaacgccaatcagcaacgactgtttgcccgccagttgttgtgccacgcggttgggaatgtaattcagctccgccatcgccgcttccactttttcccgcgttttcgcagaaacgtggctggcctggttcaccacgcgggaaacggtctgataagagacaccggcatactctgcgacatcgtataacgttactggtttcacattcaccaccctgaattgactctcttccgggcgctatcatgccataccgcgaaaggttttgcgccattcgatggtgtccgggatctcgacgctctcccttatgcgactcctgcattaggaagcagcccagtagtaggttgaggccgttgagcaccgccgccgcaaggaatggtgcatgcaaggagatggcgcccaacagtcccccggccacggggcctgccaccatacccacgccgaaacaagcgctcatgagcccgaagtggcgagcccgatcttccccatcggtgatgtcggcgatataggcgccagcaaccgcacctgtggcgccggtgatgccggccacgatgcgtccggcgtagaggatcg

SEQ ID NO: 28 - DNA, 310 bp, Artificial Sequence
  PCR product (T7 pol template)
catcggtgatgtcggcgatataggcgccagcaaccgcacctgtggcgccggtgatgccggccacgatgcgtccggcgtagaggatcgagatctcgatcccgcgaaattaatacgactcactataggggaattgtgagcggataacaattcccctctagttacaacctactacctcgcatgggtcatcaccatcatcatcacgggtccctgcaggactcagaagtcaatcaagaagctaagccagaggtcaagccagaagtcaagcctgagactcacatcaatttaaaggtgtccgatggatcttcagaga